European Patent Application EP 4 464 788 A1, published November 20, 2024. Title: System and method for checking the ability of a protein of interest to act as a substrate for an enzyme. Applicant: Julius-Maximilians-Universitaet Wuerzburg. Application EP. The sequence listing filed with the application follows.

SEQUENCE LISTING (23 sequences)

SEQ ID NO: 1 - protein, 170 aa, synthetic construct
VFTLEDFVGDWRQTAGYNLDQVLEQGGVSSLFQNLGVSVTPIQRIVLSGENGLKIDIHVIIPYEGLSGDQMGQIEKIFKVVYPVDDHHFKVILHYGTLVIDGVTPNMIDYFGRPYEGIAVFDGKKITVTGTLWNGNKIIDERLINPDGSLLFRVTINGVTGWRLCERILA

SEQ ID NO: 2 - protein, 11 aa, synthetic construct
VSGWRLFKKIS

SEQ ID NO: 3-5 - skipped (3 entries)

SEQ ID NO: 6 - DNA, 30 bp, synthetic construct
  source 1..30: mol_type = other DNA
gaattcgggagctccggtgggagctccggt

SEQ ID NO: 7 - DNA, 30 bp, synthetic construct
  source 1..30: mol_type = other DNA
acgcgtgggagctccggtgggagctccggt

SEQ ID NO: 8 - DNA, 30 bp, synthetic construct
  source 1..30: mol_type = other DNA
gggagctccggtgggagctccggtacgcgt

SEQ ID NO: 9 - DNA, 951 bp, synthetic construct
  source 1..951: mol_type = other DNA
atgccccggagggcggagaactgggacgaggccgaggtaggcgcggaggaggcaggcgtcgaagagtacggccctgaagaagacggcggggaggagtcgggcgccgaggagtccggcccggaagagtccggcccggaggaactgggcgccgaggaggagatggaggccgggcggccgcggcccgtgctgcgctcggtgaactcgcgcgagccctcccaggtcatcttctgcaatcgcagtccgcgcgtcgtgctgcccgtatggctcaacttcgacggcgagccgcagccctacccaacgctgccgcctggcacgggccgccgcatccacagctaccgaggtcacctttggctcttcagagatgcagggacacacgatgggcttctggttaaccaaactgaattatttgtgccatctctcaatgttgacggacagcctatttttgccaatatcacactgccagtgtatactctgaaagagcgatgcctccaggttgtccggagcctagtcaagcctgagaattacaggagactggacatcgtcaggtcgctctacgaagatctggaagaccacccaaatgtgcagaaagacctggagcggctgacacaggagcgcattgcacatcaacggatgggagatgaattcgggagctccggtgggagctccggtatcctctggcatgagatgtggcatgaaggcctggaagaggcatctcgtttgtactttggggaaaggaacgtgaaaggcatgtttgaggtgctggagcccttgcatgctatgatggaacggggcccccagactctgaaggaaacatcctttaatcaggcctatggtcgagatttaatggaggcccaagagtggtgcaggaagtacatgaaatcagggaatgtcaaggacctcacccaagcctgggacctctattatcatgtgttccgacgaatctcaaagtga

SEQ ID NO: 10 - DNA, 1638 bp, synthetic construct
  source 1..1638: mol_type = other DNA
atggccggcgaaggagatcagcaggacgctgcgcacaacatgggcaaccacctgccgctcctgcctgcagagagtgaggaagaagatgaaatggaagttgaagaccaggatagtaaagaagccaaaaaaccaaacatcataaattttgacaccagtctgccgacatcacatacatacctaggtgctgatatggaagaatttcatggcaggactttgcacgatgacgacagctgtcaggtgattccagttcttccacaagtgatgatgatcctgattcccggacagacattacctcttcagctttttcaccctcaagaagtcagtatggtgcggaatttaattcagaaagatagaacctttgctgttcttgcatacagcaatgtacaggaaagggaagcacagtttggaacaacagcagagatatatgcctatcgagaagaacaggattttggaattgagatagtgaaagtgaaagcaattggaagacaaaggttcaaagtccttgagctaagaacacagtcagatggaatccagcaagctaaagtgcaaattcttcccgaatgtgtgttgccttcaaccatgtctgcagttcaattagaatccctcaataagtgccagatatttccttcaaaacctgtctcaagagaagaccaatgttcatataaatggtggcagaaataccagaagagaaagtttcattgtgcaaatctaacttcatggcctcgctggctgtattccttatatgatgctgagaccttaatggacagaatcaagaaacagctacgtgaatgggatgaaaatctaaaagatgattctcttccttcaaatccaatagatttttcttacagagtagctgcttgtcttcctattgatgatgtattgagaattcagctccttaaaattggcagtgctatccagcgacttcgctgtgaattagacattatgaataaatgtacttccctttgctgtaaacaatgtcaagaaacagaaataacaaccaaaaatgaaatattcagtttatccttatgtgggccgatggcagcttatgtgaatcctcatggatatgtgcatgagacacttactgtgtataaggcttgcaacttgaatctgataggccggccttctacagaacacagctggtttcctgggtatgcctggactgttgcccagtgtaagatctgtgcaagccatattggatggaagtttacggccaccaaaaaagacatgtcacctcaaaaattttggggcttaacgcgatctgctctgttgcccacgatcccagacactgaagatgaaataagtccagacaaagtaatactttgcttgacgcgtgggagctccggtgggagctccggtatcctctggcatgagatgtggcatgaaggcctggaagaggcatctcgtttgtactttggggaaaggaacgtgaaaggcatgtttgaggtgctggagcccttgcatgctatgatggaacggggcccccagactctgaaggaaacatcctttaatcaggcctatggtcgagatttaatggaggcccaagagtggtgcaggaagtacatgaaatcagggaatgtcaaggacctcacccaagcctgggacctctattatcatgtgttccgacgaatctcaaagtga

SEQ ID NO: 11 - DNA, 285 bp, Homo sapiens
  source 1..285: mol_type = other DNA
atgatcctctggcatgagatgtggcatgaaggcctggaagaggcatctcgtttgtactttggggaaaggaacgtgaaaggcatgtttgaggtgctggagcccttgcatgctatgatggaacggggcccccagactctgaaggaaacatcctttaatcaggcctatggtcgagatttaatggaggcccaagagtggtgcaggaagtacatgaaatcagggaatgtcaaggacctcacccaagcctgggacctctattatcatgtgttccgacgaatctcaaagtga

SEQ ID NO: 12 - DNA, 1896 bp, synthetic construct
  source 1..1896: mol_type = other DNA
atggcgacggaggagaagaagcccgagaccgaggccgccagagcacagccaaccccttcgtcatccgccactcagagcaagcctacacctgtgaagccaaactatgctctaaagttcacccttgctggccacaccaaagcagtgtcctccgtgaaattcagcccgaatggagagtggctggcaagttcatctgctgataaacttattaaaatttggggcgcgtatgatgggaaatttgagaaaaccatatctggtcacaagctgggaatatccgatgtagcctggtcgtcagattctaaccttcttgtttctgcctcagatgacaaaaccttgaagatatgggacgtgagctcgggcaagtgtctgaaaaccctgaagggacacagtaattatgtcttttgctgcaacttcaatccccagtccaaccttattgtctcaggatcctttgacgaaagcgtgaggatatgggatgtgaaaacagggaagtgcctcaagactttgccagctcactcggatccagtctcggccgttcattttaatcgtgatggatccttgatagtttcaagtagctatgatggtctctgtcgcatctgggacaccgcctcaggccagtgcctgaagacgctcatcgatgacgacaacccccccgtgtcttttgtgaagttctccccgaacggcaaatacatcctggccgccacgctggacaacactctgaagctctgggactacagcaaggggaagtgcctgaagacgtacactggccacaagaatgagaaatactgcatatttgccaatttctctgttactggtgggaagtggattgtgtctggctcagaggataaccttgtttacatctggaaccttcagacgaaagagattgtacagaaactacaaggccacacagatgtcgtgatctcaacagcttgtcacccaacagaaaacatcatcgcctctgctgcgctagaaaatgacaaaacaattaaactgtggaagagtgactgcgaattcgggagctccggtgggagctccggtgtcttcacactcgaagatttcgttggggactggcgacagacagccggctacaacctggaccaagtccttgaacagggaggtgtgtccagtttgtttcagaatctcggggtgtccgtaactccgatccaaaggattgtcctgagcggtgaaaatgggctgaagatcgacatccatgtcatcatcccgtatgaaggtctgagcggcgaccaaatgggccagatcgaaaaaatttttaaggtggtgtaccctgtggatgatcatcactttaaggtgatcctgcactatggcacactggtaatcgacggggttacgccgaacatgatcgactatttcggacggccgtatgaaggcatcgccgtgttcgacggcaaaaagatcactgtaacagggaccctgtggaacggcaacaaaattatcgacgagcgcctgatcaaccccgacggctccctgctgttccgagtaaccatcaacggagtgaccggctggcggctgtgcgaacgcattctggcggggagctccggtgggagctccggtacgcgtggagtgcaggtggaaaccatctccccaggagacgggcgcaccttccccaagcgcggccagacctgcgtggtgcactacaccgggatgcttgaagatggaaagaaatttgattcctcccgggacagaaacaagccctttaagtttatgctaggcaagcaggaggtgatccgaggctgggaagaaggggttgcccagatgagtgtgggtcagagagccaaactgactatatctccagattatgcctatggtgccactgggcacccaggcatcatcccaccacatgccactctcgtcttcgatgtggagcttctaaaactggaatga

SEQ ID NO: 13 - protein, 107 aa, Homo sapiens
GVQVETISPGDGRTFPKRGQTCVVHYTGMLEDGKKFDSSRDRNKPFKFMLGKQEVIRGWEEGVAQMSVGQRAKLTISPDYAYGATGHPGIIPPHATLVFDVELLKLE

SEQ ID NO: 14 - protein, 107 aa, synthetic construct
GVQVETISPGDGRTFPRRGQTCVVHYTGMLEDGRRFDSSRDRNRPFRFMLGRQEVIRGWEEGVAQMSVGQRARLTISPDYAYGATGHPGIIPPHATLVFDVELLRLE

SEQ ID NO: 15 - protein, 170 aa, synthetic construct
VFTLEDFVGDWRQTAGYNLDQVLEQGGVSSLFQNLGVSVTPIQRIVLSGENGLRIDIHVIIPYEGLSGDQMGQIERIFRVVYPVDDHHFRVILHYGTLVIDGVTPNMIDYFGRPYEGIAVFDGRRITVTGTLWNGNRIIDERLINPDGSLLFRVTINGVTGWRLCERILA

SEQ ID NO: 16 - protein, 91 aa, Arabidopsis thaliana
KRDHHHHHHQDKKTMMMNEEDDGNGMDELLAVLGYKVRSSEMADVAQKLEQLEVMMSNVQEDDLSQLATETVHYNPAELYTWLDSMLTDLN

SEQ ID NO: 17 - protein, 344 aa, Arabidopsis thaliana
AASDEVNLIESRTVVPLNTWVLISNFKVAYNILRRPDGTFNRHLAEYLDRKVTANANPVDGVFSFDVLIDRRINLLSRVYRPAYADQEQPPSILDLEKPVDGDIVPVILFFHGGSFAHSSANSAIYDTLCRRLVGLCKCVVVSVNYRRAPENPYPCAYDDGWIALNWVNSRSWLKSKKDSKVHIFLAGDSSGGNIAHNVALRAGESGIDVLGNILLNPMFGGNERTESEKSLDGKYFVTVRDRDWYWKAFLPEGEDREHPACNPFSPRGKSLEGVSFPKSLVVVAGLDLIRDWQLAYAEGLKKAGQEVKLMHLEKATVGFYLLPNNNHFHNVMDEISAFVNAEC

SEQ ID NO: 18 - protein, 296 aa, synthetic construct
AEIGTGFPFDPHYVEVLGERMHYVDVGPRDGTPVLFLHGNPTSSYVWRNIIPHVAPTHRCIAPDLIGMGKSDKPDLGYFFDDHVRFMDAFIEALGLEEVVLVIHDWGSALGFHWAKRNPERVKGIAFMEFIRPIPTWDEWPEFARETFQAFRTTDVGRKLIIDQNVFIEGTLPMGVVRPLTEVEMDHYREPFLNPVDREPLWRFPNELPIAGEPANIVALVEEYMDWLHQSPVPKLLFWGTPGVLIPPAEAARLAKSLPNCKAVDIGPGLNLLQEDNPDLIGSEIARWLSTLEISG

SEQ ID NO: 19 - protein, 181 aa, synthetic construct
DKDCEMKRTTLDSPLGKLELSGCEQGLHRIIFLGKGTSAADAVEVPAPAAVLGGPEPLMQATAWLNAYFHQPEAIEEFPVPALHHPVFQQESFTRQVLWKLLKVVKFGEVISYSHLAALAGNPAATAAVKTALSGNPVPILIPCHRVVQGDLDVGGYEGGLAVKEWLLAHEGHRLGKPGLG

SEQ ID NO: 20 - protein, 298 aa, Arabidopsis thaliana
VPLYGFTSICGRRPEMEDAVSTIPRFLQSSSGSMLDGRFDPQSAAHFFGVYDGHGGSQVANYCRERMHLALAEEIAKEKPMLCDGDTWLEKWKKALFNSFLRVDSEIESVAPETVGSTSVVAVVFPSHIFVANCGDSRAVLCRGKTALPLSVDHKPDREDEAARIEAAGGKVIQWNGARVFGVLAMSRSIGDRYLKPSIIPDPEVTAVKRVKEDDCLILASDGVWDVMTDEEACEMARKRILLWHKKNAVAGDASLLADERRKEGKDPAAMSAAEYLSKLAIQRGSKDNISVVVVDLK

SEQ ID NO: 21 - protein, 176 aa, Arabidopsis thaliana
QDEFTQLSQSIAEFHTYQLGNGRCSSLLAQRIHAPPETVWSVVRRFDRPQIYKHFIKSCNVSEDFEMRVGCTRDVNVISGLPANTSRERLDLLDDDRRVTGFSITGGEHRLRNYKSVTTVHRFEKEEEEERIWTVVLESYVVDVPEGNSEEDTRLFADTVIRLNLQKLASITEAMN

SEQ ID NO: 22 - protein, 190 aa, synthetic construct
PSELTPEERSELKNSIAEFHTYQLDPGSCSSLHAQRIHAPPELVWSIVRRFDKPQTHRHFIKSCSVEQNFEMRVGCTRDIIVISGLPANTSTERLDILDDERRVTGASIIGGEHRLTNYKGVTTVHRFEKENRIWTVVLESYVVDMPEGNSEDDTRMLADTVVKLNLQKLATVAEAMARNSGDGSGSQVT

SEQ ID NO: 23 - protein, 158 aa, Escherichia coli
ISLIAALAVDRVIGMENAMPWNLPADLAWFKRNTLNKPVIMGRHTWESIGRPLPGRKNIILSSQPGTDDRVTWVKSVDEAIAACGDVPEIMVIGGGRVYEQFLPKAQKLYLTHIDAEVEGDTHFPDYEPDDWESVFSEFHDADAQNSHSYCFEILERR